European Patent Application EP 4 715 047 A1, published March 25, 2026. Title: 신규한 PET 분해 효소 및 그 용도. Applicant: 주식회사 자이엔. Application KR. The sequence listing filed with the application follows.

SEQUENCE LISTING (17 sequences)

SEQ ID NO: 1 - protein, 299 aa, Cryptosporangium aurantiacum
  source 1..299: note = CaPETase WT
MLSFLRSTGRPERRRASLPALLLFTAALVASGLTAAPAAQAADNPYQRGPDPTNASIEAATGPFAVGTQPIVGASGFGGGQIYYPTDTSQTYGAVVIVPGFISVWAQLNWLGPRLASQGFVVIGIETSVITDLPDPRGDQALAALDWATTRSPVASRIDRTRLAAAGWSMGGGGLRRAALQRPSLKAIVGMAPWNGERNWSAVTVPTLFFGGSSDAVASPNDHAKPFYNSITRAEKDYIELRNADHFFPTSANTTMAKYFISWLKRWVDNDTRYTQFLCPGPSTGLFAPVSASMNTCPF

SEQ ID NO: 2 - DNA, 900 bp, Cryptosporangium aurantiacum
  source 1..900: mol_type = genomic DNA; note = CaPETase WT
gtgctgtcctttctccgaagtaccggccgccccgagcgccgacgagcgtcgttaccggcgctcctgttgttcaccgctgcgctcgtcgcgagcgggctcaccgccgcccccgccgcgcaggcggccgacaacccctaccaacgcggtccggaccccacgaacgcgagtatcgaggcggcgaccggcccgttcgcggtcggcacgcagccgatcgtcggtgcctccggcttcggcggcggccagatctactacccgaccgacaccagccagacgtacggggcggtcgtgatcgtgccgggcttcatctcggtctgggcccagctcaactggctcgggccgcgcctggcgtcccagggttttgtggtcatcggcatcgagaccagcgtgatcaccgacctgcccgacccgcgcggtgaccaggcgctggccgcgctggactgggcgacgacccggagcccggtcgcgagccggatcgaccggacccggctggccgcggccggctggtcgatgggcggcggcggcctgcggcgggccgcactgcaacgcccgtcgctcaaggcgatcgtcgggatggcgccctggaacggcgagcgcaactggtccgccgtcaccgtgccgacgctgttcttcggtggttcgtccgacgccgtcgcctcgccgaacgaccacgcgaagccgttctacaacagcatcacccgagccgagaaggattacatcgaactccggaacgccgaccatttcttccccacgtcggcgaacaccacgatggcgaaatacttcatctcgtggctcaagcgttgggtggacaacgacacccgctacacccagttcctctgccccggaccgtccaccggattgttcgccccggtgagcgcgtcgatgaacacctgcccgttctga

SEQ ID NO: 3 - protein, 299 aa, synthetic construct
  source 1..299: note = CaPETaseM1
MLSFLRSTGRPERRRASLPALLLFTAALVASGLTAAPAAQAADNPYQRGPDPTNASIEAATGPFAVGTQPIVGASGFGGGQIYYPTDTSQTYGAVVIVPGFISVWAQLNWLGPRLASQGFVVIGIETSTITDLPDPRGDQALAALDWATTRSPVASRIDRTRLAAAGWSMGGGGLRRAALQRPSLKAIVGMAPWNGERNWSAVTVPTLFFGGSSDAVASPNDHAKPFYNSITRAEKDYIELRNADHFFPTSANTTMAKYFISWLKRWVDNDTRYTQFLCPGPSTGLFAPVSASMNTCPF

SEQ ID NO: 4 - protein, 299 aa, synthetic construct
  source 1..299: note = CaPETaseM2
MLSFLRSTGRPERRRASLPALLLFTAALVASGLTAAPAAQAADNPYQRGPDPTNASIEAATGPFAVGTQPIVGASGFGGGQIYYPTDTSQTYGAVVIVPGFISVWAQLNWLGPRLASQGFVVIGIETSVITDLPDPRGDQALAALDWATTRSPVASRIDRTRLAAAGWSMGGGGLRRAALQRPSLKAIVGMAPWNTERNWSAVTVPTLFFGGSSDAVASPNDHAKPFYNSITRAEKDYIELRNADHFFPTSANTTMAKYFISWLKRWVDNDTRYTQFLCPGPSTGLFAPVSASMNTCPF

SEQ ID NO: 5 - protein, 299 aa, synthetic construct
  source 1..299: note = CaPETaseM3
MLSFLRSTGRPERRRASLPALLLFTAALVASGLTAAPAAQAADNPYQRGPDPTNASIEAATGPFAVGTQPIVGASGFGGGQIYYPTDTSQTYGAVVIVPGFISVWAQLNWLGPRLASQGFVVIGIETSVITDLPDPRGDQALAALDWATTRSPVASRIDRTRLAAAGWSMGGGGLRRAALQRPSLKAIVGMAPWNGEKNWSAVTVPTLFFGGSSDAVASPNDHAKPFYNSITRAEKDYIELRNADHFFPTSANTTMAKYFISWLKRWVDNDTRYTQFLCPGPSTGLFAPVSASMNTCPF

SEQ ID NO: 6 - protein, 299 aa, synthetic construct
  source 1..299: note = CaPETaseM4
MLSFLRSTGRPERRRASLPALLLFTAALVASGLTAAPAAQAADNPYQRGPDPTNASIEAATGPFAVGTQPIVGASGFGGGQIYYPTDTSQTYGAVVIVPGFISVWAQLNWLGPRLASQGFVVIGIETSTITDLPDPRGDQALAALDWATTRSPVASRIDRTRLAAAGWSMGGGGLRRAALQRPSLKAIVGMAPWNTERNWSAVTVPTLFFGGSSDAVASPNDHAKPFYNSITRAEKDYIELRNADHFFPTSANTTMAKYFISWLKRWVDNDTRYTQFLCPGPSTGLFAPVSASMNTCPF

SEQ ID NO: 7 - protein, 299 aa, synthetic construct
  source 1..299: note = CaPETaseM5
MLSFLRSTGRPERRRASLPALLLFTAALVASGLTAAPAAQAADNPYQRGPDPTNASIEAATGPFAVGTQPIVGASGFGGGQIYYPTDTSQTYGAVVIVPGFISVWAQLNWLGPRLASQGFVVIGIETSTITDLPDPRGDQALAALDWATTRSPVASRIDRTRLAAAGWSMGGGGLRRAALQRPSLKAIVGMAPWNGEKNWSAVTVPTLFFGGSSDAVASPNDHAKPFYNSITRAEKDYIELRNADHFFPTSANTTMAKYFISWLKRWVDNDTRYTQFLCPGPSTGLFAPVSASMNTCPF

SEQ ID NO: 8 - protein, 299 aa, synthetic construct
  source 1..299: note = CaPETaseM6
MLSFLRSTGRPERRRASLPALLLFTAALVASGLTAAPAAQAADNPYQRGPDPTNASIEAATGPFAVGTQPIVGASGFGGGQIYYPTDTSQTYGAVVIVPGFISVWAQLNWLGPRLASQGFVVIGIETSVITDLPDPRGDQALAALDWATTRSPVASRIDRTRLAAAGWSMGGGGLRRAALQRPSLKAIVGMAPWNTEKNWSAVTVPTLFFGGSSDAVASPNDHAKPFYNSITRAEKDYIELRNADHFFPTSANTTMAKYFISWLKRWVDNDTRYTQFLCPGPSTGLFAPVSASMNTCPF

SEQ ID NO: 9 - protein, 299 aa, synthetic construct
  source 1..299: note = CaPETaseM7
MLSFLRSTGRPERRRASLPALLLFTAALVASGLTAAPAAQAADNPYQRGPDPTNASIEAATGPFAVGTQPIVGASGFGGGQIYYPTDTSQTYGAVVIVPGFISVWAQLNWLGPRLASQGFVVIGIETSTITDLPDPRGDQALAALDWATTRSPVASRIDRTRLAAAGWSMGGGGLRRAALQRPSLKAIVGMAPWNTEKNWSAVTVPTLFFGGSSDAVASPNDHAKPFYNSITRAEKDYIELRNADHFFPTSANTTMAKYFISWLKRWVDNDTRYTQFLCPGPSTGLFAPVSASMNTCPF

SEQ ID NO: 10 - DNA, 33 bp, synthetic construct
  source 1..33: mol_type = other DNA
tatatcatatggcggccgacaacccctaccaac

SEQ ID NO: 11 - DNA, 33 bp, synthetic construct
  source 1..33: mol_type = other DNA
tatatctcgaggaacgggcaggtgttcatcgac

SEQ ID NO: 12 - DNA, 34 bp, synthetic construct
  source 1..34: mol_type = other DNA
tatacatatgcgcggtccgaatccgacagccgcc

SEQ ID NO: 13 - DNA, 34 bp, synthetic construct
  source 1..34: mol_type = other DNA
gcgcctcgaggctgcaattcgctgtacgaaaatc

SEQ ID NO: 14 - DNA, 30 bp, synthetic construct
  source 1..30: mol_type = other DNA
gcgccatatggccaacccctacgaacgtgg

SEQ ID NO: 15 - DNA, 27 bp, synthetic construct
  source 1..27: mol_type = other DNA
gcgcctcgaggaatgggcaggtcgagc

SEQ ID NO: 16 - DNA, 34 bp, synthetic construct
  source 1..34: mol_type = other DNA
tatatcatatgcaatccaacccgtaccagcgcgg

SEQ ID NO: 17 - DNA, 33 bp, synthetic construct
  source 1..33: mol_type = other DNA
tatatctcgagctggcagtggcggttgttcgtc